European Patent Application EP 4 227 685 A2, published August 16, 2023. Title: PROTEINS AND NUCLEIC ACIDS USEFUL IN VACCINES TARGETING STAPHYLOCOCCUS AUREUS. Applicant: Evaxion Biotech A/S. The sequence listing filed with the application follows.

SEQUENCE LISTING (53 sequences)

SEQ ID NO: 1 - protein, 140 aa, Staphylococcus aureus
MAKGNLFKAILGIGGAVAAVLVTRKDSRDKLKAEYNKYKQDPQSYKDNAKDKATQLGTIANETIKEVKTNPKEYANRLKNNPKAFFEEEKSKFTEYDNKTDESIEKGKFDDEGGAAPNNNLRIVTEEDLKKNKNALSDKE

SEQ ID NO: 2 - protein, 193 aa, Staphylococcus aureus
MKKLVSIVGATLLLAGCGSQNLAPLEEKTTDLREDNHQLKLDIQELNQQISDSKSKIKGLEKDKENSKKTASNNTKIKLMNVTSTYYDKVAKALKSYNDIEKDVSKNKGDKNVQSKLNQISNDIQSAHTSYKDAIDGLSLSDDDKKTSKNIDKLNSDLNHAFDDIKNGYQNKDKKQLTKGQQALSKLNLNAKS

SEQ ID NO: 3 - protein, 209 aa, Staphylococcus aureus
MKKLVTGLLALSLFLAACGQDSDQQKDSNKEKDDKAKTEQQDKKTNDSSKDKKDNKDDSKDVNKDNKDNSANDNQQQSNSNATNNDQNQTNNNQSNSGQTTNNQKSSYVAPYYGQNAAPVARQIYPFNGNKSQALQQLPNFQTALNAANNEANKFGNGHKVYNDYSIEEHNGNYKYVFSFKDPNVNGKYSIVTVDYTGQAMVTDPNYQQ

SEQ ID NO: 4 - protein, 242 aa, Staphylococcus aureus
MKKVMGILLASTLILGACGHHQDSAKKESTSHKKKENDNEELNEELKEFKSKKNMDIKIKGDTIVSDKFEAKIKEPFIINEKDEKKKYIAFKMEITAKKDDKDLNPSSISHDYINITQDDKNTVNKLRDGYLLSDKNYKDWTEHNQDQIKKGKTAQAMFIYELRGDGNINLNVHKYSEDKTVDSKSFKFSKLKTEDFSHRAETREEVEKKEKEFEEEYKKEQEREKEKEKQKDDDHSGLDEV

SEQ ID NO: 5 - protein, 327 aa, Staphylococcus aureus
MKKWQFVGTTALGATLLLGACGGGNGGSGNSDLKGEAKGDGSSTVAPIVEKLNEKWAQDHSDAKISAGQAGTGAGFQKFIAGDIDFADASRPIKDEEKQKLQDKNIKYKEFKIAQDGVTVAVNKENDFVDELDKQQLKAIYSGKAKTWKDVNSKWPDKKINAVSPNSSHGTYDFFENEVMNKEDIKAEKNADTNAIVSSVTKNKEGIGYFGYNFYVQNKDKLKEVKIKDENGKATEPTKKTIQDNSYALSRPLFIYVNEKALKDNKVMSEFIKFVLEDKGKAAEEGGYVAAPEKTYKSQLDDLKAFIDKNQKSDDKKSDDKKSEDKK

SEQ ID NO: 6 - protein, 357 aa, Staphylococcus aureus
MKGKFLKVSSLFVATLTTATLVSSPAANALSSKAMDNHPQQTQTDKQQTPKIQKGGNLKPLEQRERANVILPNNDRHQITDTTNGHYAPVTYIQVEAPTGTFIASGVVVGKDTLLTNKHIVDATHGDPHALKAFASAINQDNYPNGGFTAEQITKYSGEGDLAIVKFSPNEQNKHIGEVVKPATMSNNAETQVNQNITVTGYPGDKPVATMWESKGKITYLKGEAMQYDLSTTGGNSGSPVFNEKNEVIGIHWGGVPNQFNGAVFINENVRNFLKQNIEDINFANDDHPNNPDNPDNPNNPDNPNNPDNPNNPDNPDNPNNPDNPNNPDNPNNPDQPNNPNNPDNGDNNNSDNPDAA

SEQ ID NO: 7 - protein, 399 aa, Staphylococcus aureus
MKRTLVLLITAIFILAACGNHKDDQAGKDNQKHNNSSNQVKEIATDKNVQGDNYRTLLPFKESQARGLLQDNMANSYNGGDFEDGLLNLSKEVFPTDKYLYQDGQFLDKKTINAYLNLKYTKREIDKMSEKDKKDKKANENLGLNPSHEGETDPEKIAEKSPAYLSNILEQDFYGGGDTKGKNIKGMTIGLAMNSVYYYKKEKDGPTFSKKLDDSEVKKQGKQMASEILSRLRENDDLKDIPIHFAIYKQSSEDSITPGEFITQATAEKSQTKLNEWHNINEKSALLPSSTAADYDENLNNNFKQFNDNLQSYFSNFTQAVGKVKFVDKKPQRLVVDLPIDYYGQAETIGITQYVTEQANKYFDKIDNYEIRIKDGNQPRALISKTKDDKEPQVHIYSN

SEQ ID NO: 8 - protein, 495 aa, Staphylococcus aureus
MRENFKLRKMKVGLVSVAITMLYIMTNGQAEASEANEKPSTNQESKVVSQTEQNSKETKTVESNKNFVKLDTIKPGAQKITGTTLPNHYVLLTVDGKSADSVENGGLGFVEANDKGEFEYPLNNRKIVHNQEIEVSSSSPDLGEDEEDEEVEEASTDKAGVEEESTEAKVTYTTPRYEKAYEIPKEQLKEKDGHHQVFIEPITEGSGIIKGHTSVKGKVALSINNKFINFEESVKGGVSKEDTKASSDGIWMPIDDKGYFNFDFKTKRFDNLELKEGNDISLTFAPDDEEDALKPLIFKTKVTSLEDIDKAETKYDHTKLNKVKVLDNVKEDLHVDEIYGSLYHTDKGKGILDKEGTKVIKGKTKFANAVVKVDSELGEAQLFPDLQVNEKGEFSFDSHGAGFRLQNGEKLNFTVVDPITGDLLSNEFVSKEIDIEETPEQKADREFDEKLENTPAYYKLYGDKIVGFDTNDFPITWFYPLGEKKVERTTPKLEK

SEQ ID NO: 9 - protein, 507 aa, Staphylococcus aureus
MSKKLKIIIPIIIVLLLIGGIAWGVYAFFANTPKNTYLKSEQQTAKMYKDYFNDRFENEVKFQEKMKDNSFLSSLELSADASDEIVKGLGIPKSVVNASKIKMSYGHDPKKEKSMINLEPTIADSALGKFQLAADKDKHYFESPLFKGKYSVNNSDLLSTYSKLTGEDEETAKENGITNQQLNLNTLFSNAQAQQSDYSKIAEKYSELIVDKLDDDNFDKGKKEEIKVNGEKYKVRPVTLTLSRADTKKITLAVLEEAKKDKDLKKLMEEQGTTKDFEKDIKKAIDDVKETKKDEFAKIQSKIYTEKHTIVKREITITDKENNKTKIKGTNTLEDDKLKLDYALDFDQDKYTYAEAKYTIKGVSSKEKDNKYSDKYEFGKKTEYDESKIKLDNQEKVDGTKRQDKGKITVALDKYSDENEFTFENNIDSDVKNNTQKSTLNIGIKYAEEPINFILKSSTKLKADIDFDDSGAKDFNSLSSKDREKLEKEIEKNGGKMFESILKKASK

SEQ ID NO: 10 - protein, 509 aa, Staphylococcus aureus
MRKFSRYAFTSMATVTLLSSLTPAALASDTNHKPATSDINFEITQKSDAVKALKELPKSENVKNHYQDYSVTDVKTDKKGFTHYTLQPSVDGVHAPDKEVKVHADKSGKVVLINGDTDAKKVKPTNKVTLSKDEAADKAFNAVKIDKNKAKNLQDDVIKENKVEIDGDSNKYIYNIELITVTPEISHWKVKIDADTGAVVEKTNLVKEAAATGTGKGVLGDTKDININSIDGGFSLEDLTHQGKLSAYNFNDQTGQATLITNEDENFVKDDQRAGVDANYYAKQTYDYYKNTFGRESYDNHGSPIVSLTHVNHYGGQDNRNNAAWIGDKMIYGDGDGRTFTNLSGANDVVAHELTHGVTQETANLEYKDQSGALNESFSDVFGYFVDDEDFLMGEDVYTPGKEGDALRSMSNPEQFGQPSHMKDYVYTEKDNGGVHTNSGIPNKAAYNVIQAIGKSKSEQIYYRALTEYLTSNSNFKDCKDALYQAAKDLYDEQTAEQVYEAWNEVGVE

SEQ ID NO: 11 - protein, 515 aa, Staphylococcus aureus
MKKKLGMLLLVPAVTLSLAACGNDDGKDKDGKVTIKTTVYPLQSFAEQIGGKHVKVSSIYPAGTDLHSYEPTQKDILSASKSDLFMYTGDNLDPVAKKVASTIKDKDKKLSLEDKLDKAKLLTDQHEHGEEHEHEGHDHGKEEHHHHGGYDPHVWLDPKINQTFAKEIKDELVKKDPKHKDDYEKNYKKLNDDLKKIDNDMKQVTKDKQGNAVFISHESIGYLADRYGFVQKGIQNMNAEDPSQKELTKIVKEIRDSNAKYILYEDNVANKVTETIRKETDAKPLKFYNMESLNKEQQKKDNITYQSLMKSNIENIGKALDSGVKVKDDKAESKHDKAISDGYFKDEQVKDRELSDYAGEWQSVYPYLKDGTLDEVMEHKAENDPKKSAKDLKAYYDKGYKTDITNIDIKGNEITFTKDGTKHTGKYEYNGKKTLKYPKGNRGVRFMFKLVDGNDKDLPKFIQFSDHNIAPKKAEHFHIFMGNDNDALLKEMDNWPTYYPSKLNKDQIKEEMLAH

SEQ ID NO: 12 - protein, 564 aa, Staphylococcus aureus
MVLYIILAIIVIILIAVGVLFYLRSNKRQIIEKAIERKNEIETLPFDQNLAQLSKLNLKGETKTKYDAMKKDNVESTNKYLAPVEEKIHNAEALLDKFSFNASQCEIDDANELMDSYEQSYQQQLEDVNEIIALYKDNDELYDKCKVDYREMKRDVLANRHQFGEAASLLETEIEKFEPRLEQYEVLKADGNYVQAHNHIAALNEQMKQLRSYMEEIPELIRETQKELPGQFQDLKYGCRDLKVEGYDLDHVKVDSTLQSLKTELSFVEPLISRLELEEANDKLANINDKLDDMYDLIEHEVKAKNDVEETKDIITDNLFKAKDMNYTLQTEIEYVRENYYINESDAQSVRQFENEIQSLISVYDDILKEMSKSAVRYSEVQDNLQYLEDHVTVINDKQEKLQNHLIQLREDEAEAEDNLLRVQSKKEEVYRRLLASNLTSVPERFIIMKNEIDHEVRDVNEQFSERPIHVKQLKDKVSKIVIQMNTFEDEANDVLVNAVYAEKLIQYGNRYRKDYSNVDKSLNEAERLFKNNRYKRAIEIAEQALESVEPGVTKHIEEEVIKQ

SEQ ID NO: 13 - protein, 619 aa, Staphylococcus aureus
MPKNKILIYLLSTTLVLPTLVSPTAYADTPQKDTTAKTTSHDSKKSTDDETSKDTTSKDIDKADNNNTSNQDNNDKKVKTIDDSTSDSNNIIDFIYKNLPQTNINQLLTKNKYDDNYSLTTLIQNLFNLNSDISDYEQPRNGEKSTNDSNKNSDNSIKNDTDTQSSKQDKADNQKAPKSNNTKPSTSNKQPNSPKPTQPNQSNSQPASDDKVNQKSSSKDNQSMSDSALDSILDQYSEDAKKTQKDYASQSKKDKNEKSNTKNPQLPTQDELKHKSKPAQSFNNDVNQKDTRATSLFETDPSISNNDDSGQFNVVDSKDTRQFVKSIAKDAHRIGQDNDIYASVMIAQAILESDSGRSALAKSPNHNLFGIKGAFEGNSVPFNTLEADGNQLYSINAGFRKYPSTKESLKDYSDLIKNGIDGNRTIYKPTWKSEADSYKDATSHLSKTYATDPNYAKKLNSIIKHYQLTQFDDERMPDLDKYERSIKDYDDSSDEFKPFREVSDNMPYPHGQCTWYVYNRMKQFGTSISGDLGDAHNWNNRAQYRDYQVSHTPKRHAAVVFEAGQFGADQHYGHVAFVEKVNSDGSIVISESNVKGLGIISHRTINAAAAEELSYITGK

SEQ ID NO: 14 - protein, 681 aa, Staphylococcus aureus
MMKSQNKYSIRKFSVGASSILIATLLFLSGGQAQAAEKQVNMGNSQEDTVTAQSIGDQQTRENANYQRENGVDEQQHTENLTKNLHNDKTISEENHRKTDDLNKDQLKDDKKSSLNNKNIQRDTTKNNNANPRDVNQGLEQAINDGKQSKVASQQQSKEADNSQDLNANNNLPSQSRTKVSPSLNKSDQTSQREIVNETEIEKVQPQQKNQANDKITDHNFNNEQEVKPQKDEKTLSVSDLKNNQKSPVEPTKDNDKKNGLNLLKSSAVATLPNKGTKELTAKAKGDQTNKVAKQGQYKNQDPIVLVHGFNGFTDDINPSVLAHYWGGNKMNIRQDLEENGYKAYEASISAFGSNYDRAVELYYYIKGGRVDYGAAHAAKYGHERYGKTYEGIYKDWKPGQKVHLVGHSMGGQTIRQLEELLRNGSREEIEYQKKHSGEISPLFKGNNDNMISSITTLGTPHNGTHASDLAGNEALVRQIVFDIGKMFGNKNSRVDFGLAQWGLKQKPNESYIDYVKRVKQSNLWKSKDNGFYDLTREGATDLNRKTSLNPNIVYKTYTGEATHKALNSDRQKADLNMFFPFVITGNLIGKATEKEWRENDGLVSVISSQHPFNQAYTNATDKIQKGIWQVTPTKHDWDHVDFVGQDSSDTVRTREELQDFWHHLADDLVKTEKVTDTKQA

SEQ ID NO: 15 - protein, 806 aa, Staphylococcus aureus
MTNKMKKWQKLSTITLLMTGVIALNNGEFRNVDKHQIAVADTNVQTPDYEKLKKTWLDVNYGYDQYDENNQDMKKKFDAKEKEAKKLLDDMKTDTNRTYLWSGAENLETNSSHMTKTYRNIEKIAESMQHKNTVLKTVENKLKIKEALDWMHKNVYGKNPSQKVEDLTKNRKGQTTPKNNSLNWWDYEIGTPRALTNTLLLMDDMLTKDEMKNYSKPISTYAPSSDKILSSVGESEDAKGGNLVDISKVKLLESVIEEDVDMLKKSIDSFNKVFTYVQDSATGKGRNGFYKDGSYIDHQDVPYTGAYGVVLLEGISQMMPMIKESPFKTTQDNATLSNWIDEGFMPLIYKGEMMDLSRGRAISRENETSHTASATVMKSLLRLNDTMDDSTKTRYKQIVKTSVNSDSSYNQNNYLNSYSDIAKMKKLMNDSTISKNDLTQQLKIYNDMDRVTYHNKDLDFAFGLSMTSKNIARYENINGENLKGWHTGAGMSYLYNSDVKHYRDNFWATADMTCLPGTTTLNDMPSTNTKNDKSFVGGTKLNNKYASIGMDFENQDKTLTAKKSYFILNDKIVFLGTGIKSTDSSKNPVTSVENRKANGYKLFKDDIEITTSDVNAQETHSVFLESNDTKKNIGYHFLDKPKITVKKESHTGKWSEINKSQKKDDKKDEYYEVTQTHNTSDSKYAYVLYPGLSKSDFKSKNNNVSIVKQDEDFHVIKDNDGVFAGVNYSDNTKSFDINGITVELKEKGMFVIKKKDDKAYKCSFYNPETTNTASNIESKIFIKGYTITNKSVINSNDAGVNFELTK

SEQ ID NO: 16 - protein, 808 aa, Staphylococcus aureus
MTYRMKKWQKLSTITLLMAGVITLNGGEFRSIDKHQIAVADTNVQTTDYEKLRNIWLDVNYGYDKYDENNPDMKKKFEATENEAEKLLKEMKTESDRKYLWESSKDLDTKSADMTRTYRNIEKISEAMKHKNTKLKTDENKTKVKDALEWLHKNAYGKEPDKKVADLTSNFKNKTSRNTNLNWWDYEIGTPRALTNTLILLQEDFTDEEKKKYTAPIKTFAPDSDKILSSVGKSEPAKGGNLVDISKVKLLESIIEEDKDMMKKSIDSFNTVFTYAQNSATGKERNGFYKDGSYIDHQDVPYTGAYGVVLLEGISQMMPMIKETPFNDSNQNDTTLKSWIDDGFMPLIYKGEMMDLSRGRAISRENETSHSASATVMKSLLRLSDTMDKSTKAKYKKIVKTSVESDSSYKQTDYLSSYSDISKMKSLMEDSTISTNGLTQQLKIYNDMDRVTYHNKGLDFAFGLSMTSKNVARYESINGENLKGWHTGAGMSYLYNSDVKHYRDNFWATADMKRLAGTTTLDNEEPKSTDVKKSSKTFVGGTKFDDQHASIGMDFENQDKTLTAKKSYFILNDKIVFLGTGIKSTDSSKNPVTTIENRKANDYKLYKDDTQTTNSDNQETNSLFLESTNSTQNNIGYHFLNESKITVKKESHTGKWSDINKSQKDIQKTDEYYEVTQKHSNTDSKYAYVLYPGLSKDVFKSKASKVTVVKQEDDFHVVKDNESVWAGINYSDSAKTFEINNTKVEVKAKGMFILTKKDDNTYECSFYNPESTNSVSDIESKISMTGYSIINKNTSTSNESGVRFELTK

SEQ ID NO: 17 - DNA, 423 bp, Staphylococcus aureus
  source 1..423: mol_type = genomic DNA
atggcaaaaggtaatttatttaaagcgattttaggtataggtggcgctgtagcagctgtacttgttacacgtaaagatagtcgtgacaagctgaaagcagaatataataaatacaaacaagatcctcaaagctataaagataatgctaaggataaagcgacgcaattaggaacaattgcaaatgaaacaattaaagaagtaaaaacaaatccgaaagaatatgctaatagattaaaaaataatccaaaagcatttttcgaagaagaaaaatcaaaatttaccgaatatgacaataagactgacgaaagtattgaaaaaggtaaatttgatgatgaaggtggcgcagcaccaaataataatttacgtatcgtcactgaagaagatttaaaaaagaataaaaatgcattgtctgataaagaataa

SEQ ID NO: 18 - DNA, 582 bp, Staphylococcus aureus
  source 1..582: mol_type = genomic DNA
atgaaaaaattggtttcaattgttggcgcaacattattgttagctggatgtggatcacaaaatttagcaccattagaagaaaaaacaacagatttaagagaagataatcatcaactcaaactagatattcaagaacttaatcaacaaattagtgattctaaatctaaaattaaagggcttgaaaaggataaagaaaatagtaaaaaaactgcatctaataatacgaaaattaaattgatgaatgttacatcaacatactacgacaaagttgctaaagctttgaaatcctataacgatattgaaaaggatgtaagtaaaaacaaaggcgataagaatgttcaatcgaaattaaatcaaatttctaatgatattcaaagtgctcacacttcatacaaagatgctatcgatggtttatcacttagtgatgatgataaaaaaacgtctaaaaatatcgataaattaaactctgatttgaatcatgcatttgatgatattaaaaatggctatcaaaataaagataaaaaacaacttacaaaaggacaacaagcgttgtcaaaattaaacttaaatgcaaaatcatga

SEQ ID NO: 19 - DNA, 630 bp, Staphylococcus aureus
  source 1..630: mol_type = genomic DNA
atgaaaaaattagttacagggttattagcattatcattatttttagctgcatgtggtcaagatagtgaccaacaaaaagacagtaataaagaaaaagatgataaagcgaaaactgaacaacaagataaaaaaacaaatgattcatctaaagataagaaagacaataaagatgatagtaaagacgtaaacaaagataataaagataatagtgcaaacgataaccagcaacaatctaattcaaatgcaacaaacaatgaccaaaatcaaacgaataataaccagtcaaacagtggacaaacgactaacaatcaaaaatcaagttacgttgcaccatattatggacaaaacgcagcgccagtggctcgtcaaatttatccatttaatggtaataaatcacaagcattacaacaattgcctaatttccaaacagctttaaatgcagctaacaacgaagcaaataaatttggtaatggtcataaagtttataatgattattcaattgaagaacataatggtaactataagtatgtttttagttttaaagacccaaacgtaaatggaaaatattcaattgtaacggttgattatactggacaagcaatggttactgatccaaactaccaacaataa

SEQ ID NO: 20 - DNA, 729 bp, Staphylococcus aureus
  source 1..729: mol_type = genomic DNA
atgaaaaaagtaatggggatattattagcaagtacacttatcttaggtgcttgtggacatcatcaagatagtgcaaaaaaagagagcactagtcacaaaaagaaagaaaatgacaatgaagaattaaatgaagaacttaaagaatttaaaagcaaaaaaaatatggatataaaaattaaaggcgatactattgttagtgacaaatttgaagctaaaataaaagaaccgtttatcatcaatgaaaaagatgagaaaaagaaatatatcgcttttaaaatggaaattactgctaaaaaagacgataaagatttaaatccatcttctatttctcatgactatattaatatcactcaagatgataaaaatacagtaaataaattaagagatggttatcttttaagtgataaaaattataaagattggacagaacataaccaagatcaaattaaaaaaggcaaaactgcacaagccatgtttatctatgagttaagaggtgatggaaacattaatttaaatgtccataaatactcagaagataaaacagttgattctaaatcattcaaatttagtaaacttaaaaccgaagatttttctcatagagcggaaacaagggaagaagtagaaaagaaagaaaaagaatttgaagaagagtacaaaaaagaacaagaacgagagaaagaaaaagaaaagcaaaaagatgacgaccacagtggtttagatgaagtataa

SEQ ID NO: 21 - DNA, 984 bp, Staphylococcus aureus
  source 1..984: mol_type = genomic DNA
atgaaaaaatggcaatttgttggtactacagctttaggtgcaacactattattaggtgcttgtggtggcggtaatggtggcagtggtaatagtgatttaaaaggggaagctaaaggggatggctcatcaacagtagcaccaattgtggagaaattaaatgaaaaatgggctcaagatcactcggatgctaaaatctcagcaggacaagctggtacaggtgctggtttccaaaaattcattgcaggagatatcgacttcgctgatgcttctagaccaattaaagatgaagagaagcaaaaattacaagataagaatatcaaatacaaagaattcaaaattgcgcaagatggtgtaacggttgctgtaaataaagaaaatgattttgtagatgaattagacaaacagcaattaaaagcaatttattctggaaaagctaaaacatggaaagatgttaatagtaaatggccagataaaaaaataaatgctgtatcaccaaactcaagtcatggtacttatgacttctttgaaaatgaagtaatgaataaagaagatattaaagcagaaaaaaatgctgatacaaatgctatcgtttcttctgtaacgaaaaacaaagagggaatcggatactttggatataacttctacgtacaaaataaagataaattaaaagaagttaaaatcaaagatgaaaatggtaaagcaacagagcctacgaaaaaaacaattcaagataactcttatgcattaagtagaccattattcatttatgtaaatgaaaaagcattgaaagataataaagtaatgtcagaatttatcaaattcgtcttagaagataaaggtaaagcagctgaagaaggtggatatgtagcagcaccagagaaaacatacaaatcacaattagatgatttaaaagcatttattgataaaaatcaaaaatcagacgacaagaaatctgatgataaaaagtctgaagacaagaaataa

SEQ ID NO: 22 - DNA, 1074 bp, Staphylococcus aureus
  source 1..1074: mol_type = genomic DNA
atgaaaggtaaatttttaaaagttagttctttattcgttgcaactttgacaacagcgacacttgtgagttctccagcagcaaatgcgttatcttcaaaagctatggacaatcatccacaacaaacgcagacagacaaacagcaaacacctaagattcaaaaaggcggtaaccttaaaccattagaacaacgtgaacgcgctaatgttatattaccaaataacgatcgtcaccaaatcacagatacaacgaatggtcattatgcacctgttacttatattcaagttgaagcacctactggtacatttattgcttctggtgtagttgtaggtaaagatacacttttaacaaataaacacatcgtagatgctacgcacggtgatcctcatgctttaaaagcattcgcttctgcaattaaccaagacaattatcctaatggtggtttcactgctgaacaaatcactaaatattcaggcgaaggtgatttagcaatcgttaaattctcccctaatgagcaaaacaaacatattggcgaagtagttaaaccagcaacaatgagtaataatgctgaaacacaagttaaccaaaatattactgtaacaggatatcctggtgataaacctgtcgcaacaatgtgggaaagtaaaggaaaaataacgtacttaaaaggtgaagcaatgcaatatgatttaagtacaactggtggtaactcaggttcacctgtatttaatgaaaaaaatgaagtcattggcattcattggggtggcgttccaaatcaatttaacggtgcagtatttattaatgaaaatgtacgcaacttcttaaaacaaaatattgaagatatcaatttcgcaaatgatgaccaccctaacaaccctgataatccagacaatccaaataatccggacaatcctaacaaccctgataaccctaacaaccctgataatccagacaatcctaataatcctgataaccctaacaacccggacaatccaaataaccctgaccaacctaacaacccaaataacccggacaatggcgataacaataattcagacaaccctgacgctgcataa

SEQ ID NO: 23 - DNA, 1200 bp, Staphylococcus aureus
  source 1..1200: mol_type = genomic DNA
atgaagcgtacattagtattattgattacagctatctttatactcgctgcttgtggtaaccataaggatgaccaggctggaaaagataatcaaaaacataacaatagttcaaatcaagtaaaagaaattgctacggataaaaatgtacaaggtgataactatcgtacattgttaccatttaaagaaagccaggcaagaggacttttacaagataacatggcaaatagttataatggcggcgactttgaagatggtttattgaacttaagtaaagaagtgtttccaacagacaaatatttgtatcaagatggtcaatttttggacaagaaaacaattaatgcctatttaaatcttaagtatacaaaacgtgaaatcgataaaatgtctgaaaaagataaaaaagacaagaaagcgaatgaaaatttaggacttaatccatcacacgaaggtgaaacagatcctgaaaagattgcagaaaaatcaccagcctatttatctaacattttagagcaagatttttatggtggtggagatacaaaaggtaagaatattaaaggtatgacgattggtttagctatgaatagtgtttattactataaaaaagaaaaagatggaccgacttttagtaaaaaactagatgatagcgaagttaaaaagcaaggtaaacaaatggctagtgagatattatcaaggttacgtgaaaatgatgatttaaaagatataccaattcattttgcaatttataagcaatcaagtgaagattcaatcacaccaggtgaatttatcactcaagcgactgcagaaaagagtcaaacaaagcttaatgaatggcataatatcaatgaaaaatcagctttattaccttcttcaacagcagcagattatgatgaaaatttaaataataatttcaagcaatttaatgataatttgcaatcatatttttctaatttcacacaagcagtaggaaaagttaaatttgttgataaaaagccacaacgattagtagtagatttaccaatcgattactatggacaagctgaaacaattggtattacacagtacgttactgaacaagcgaataaatatttcgataaaatcgataactatgaaattcggattaaagatggtaaccaaccacgtgctttaattagtaagacaaaagatgacaaagaaccgcaagttcatatttacagtaattaa

SEQ ID NO: 24 - DNA, 1488 bp, Staphylococcus aureus
  source 1..1488: mol_type = genomic DNA
atgagggaaaattttaagttacgtaaaatgaaagtcgggttagtatctgttgcaattacaatgttatatatcatgacaaacggacaagcagaagcatcagaggctaatgagaagccaagtacaaatcaagaatcaaaagttgtttcacagactgaacaaaattcaaaagaaacaaaaacagtagaatctaataagaactttgttaaattagatactattaaacctggagctcaaaagataacgggaactactttaccaaatcactatgttttattaacagttgatgggaaaagtgcggattcagtagaaaatggcggtttgggttttgttgaagcaaatgacaaaggagaatttgagtaccctttaaataatcgtaaaattgttcataatcaagaaattgaggtttcgtcgtcaagccctgatttaggtgaagatgaagaagatgaagaggtggaagaagcttcaactgataaagctggcgttgaggaagaaagtacagaagctaaagttacttacacaacaccgcgatatgaaaaagcgtatgaaataccgaaagaacaactaaaagaaaaagatggacatcaccaagtttttatcgaacctattactgaaggatcaggtattattaaagggcatacgtctgtaaaaggtaaagttgctttatctattaataataaatttattaattttgaagagagcgttaagggcggagttagtaaagaagacactaaagctagttcagatggtatctggatgcctattgatgacaaaggatactttaactttgacttcaaaacgaaacgtttcgataatttagagttaaaagaaggtaatgacatttcactaacatttgcacctgatgatgaagaagatgcattaaaacctttaattttcaaaactaaagtaacgagcttagaagatatcgataaagcagaaactaaatatgaccatactaaactcaacaaagtgaaagttttagataatgttaaagaagatttacatgttgatgaaatatatggaagcttatatcatacagacaaaggtaaaggtattcttgataaagaaggtactaaagtaattaaaggaaagactaaattcgcgaatgcagtagtgaaggtagactctgaactaggtgaagcacaattattccctgatttacaagtaaatgaaaaaggtgaatttagctttgactcacatggtgctggttttagattacaaaatggagaaaaattaaacttcacagtggttgatcctattacaggtgacttgttaagtaatgagtttgtttctaaagagattgatattgaagaaacacctgaacaaaaagcggatcgtgagtttgacgaaaaacttgaaaatacgcctgcttactacaagttatacggcgataaaatagttggattcgatactaacgatttcccgattacttggttctatccattgggtgaaaagaaagttgaacgtacaacacctaaattagaaaaataa

SEQ ID NO: 25 - DNA, 1524 bp, Staphylococcus aureus
  source 1..1524: mol_type = genomic DNA
atgtctaaaaagttaaaaattataattcctattattattgtcttattattaataggtggaatcgcatggggagtttatgcattttttgcaaacacaccgaaaaatacatacttaaaaagtgaacaacaaactgcaaaaatgtataaagattattttaatgaccgttttgaaaacgaagtgaagttccaagaaaagatgaaagataattcatttttatcttcattagaattaagcgcagatgcatctgatgaaattgttaaagggcttggtattcctaaatctgttgttaatgcttcgaaaattaaaatgtcatatggacatgatcctaaaaaagagaaatcaatgattaatcttgaaccaacaatagcagactctgcattagggaaattccagttagctgcagataaagataagcattatttcgaatcaccattatttaaagggaaatatagtgttaataattctgatttattatcaacttattcaaaacttacaggtgaagatgaagaaacagcaaaagaaaatggtattacaaaccaacaactaaatttaaatactcttttcagtaatgctcaagcacaacaaagtgactacagcaaaattgccgaaaaatattccgaacttattgtcgacaaattagatgacgataattttgataaaggtaaaaaagaagaaattaaggttaatggtgaaaagtacaaagttagacctgtcacgttaacacttagcagagctgacactaaaaaaattacattagctgtattagaagaagctaaaaaggataaagaccttaaaaaattaatggaagaacaaggtactacaaaagactttgaaaaagacattaaaaaagcaattgacgatgtcaaagaaactaaaaaggatgaatttgctaaaattcaatctaaaatttataccgaaaaacatacgattgtaaaacgagaaattactattacagacaaagaaaataataaaactaaaatcaaaggtactaatactttagaagacgataagttaaaactagattacgcacttgatttcgatcaagataaatacacgtatgctgaagcgaaatatacaattaaaggcgtatcttctaaggaaaaagacaataaatacagtgataaatacgaatttggtaaaaagacagaatatgatgaatcaaaaatcaaattagataaccaagaaaaagtagatggcacaaaacgtcaagataaaggtaaaatcactgtcgcgttagataaatatagcgacgaaaatgaattcacttttgaaaataatatagattctgacgtaaaaaataacactcagaaatctacgttaaatatcggcatcaaatatgctgaagaaccaattaatttcattttaaaatctagcacaaaattgaaagcagatattgattttgatgatagtggtgcgaaagatttcaatagtctatcttcaaaagaccgtgaaaaacttgaaaaagaaatcgaaaaaaatggcggcaaaatgtttgaatcaattttaaaaaaggcatctaaataa

SEQ ID NO: 26 - DNA, 1530 bp, Staphylococcus aureus
  source 1..1530: mol_type = genomic DNA
gtgaggaaattttcaagatatgcatttacaagtatggcaacagtaacgttgctgagctctttgacacctgcagcactagcgagtgatacgaatcacaaaccagcaacttcagatattaattttgaaatcacgcaaaagagtgatgcagttaaagcattaaaagagttacctaaatctgaaaatgtgaaaaatcattatcaagattactctgttacagatgtaaaaacagataagaaaggattcacgcattacacgttacaaccgagtgtggatggtgtgcatgcgcctgacaaagaagtgaaagtgcatgcggacaaatcgggtaaagtcgttttaatcaacggtgatactgatgcgaagaaagtaaagccgacaaataaagtgacattaagcaaggatgaagcggctgacaaagcatttaacgcagttaagattgataaaaataaagctaaaaacctccaagatgacgttatcaaagaaaataaagtcgaaatcgatggtgacagtaataaatacatttacaatattgaattaattacagtaacaccagaaatttcacattggaaagttaaaattgatgcagacacaggagcagttgttgaaaaaacgaacttagttaaagaagcagcagcaactggcacaggtaaaggtgtgcttggagatacaaaagatatcaatatcaatagtattgatggtggatttagtttagaggatttgacgcatcaaggtaaattatcagcatacaattttaacgatcaaacaggtcaagcgacattaattactaatgaagatgaaaacttcgtcaaagatgatcaacgtgctggtgtagatgcgaattattatgctaaacaaacatatgattactacaaaaatacatttggtcgtgagtcttacgataaccatggtagtccaatagtctcattaacacatgtaaatcattatggtggacaagataacagaaataacgctgcatggattggagacaaaatgatttatggtgatggcgatggccgcacgtttacaaatttatcaggtgcaaatgacgtagtagcacatgagttaacacatggcgtgacacaagaaacggcgaatttagagtataaagatcaatctggtgcgttaaatgaaagcttttcagatgtttttggatactttgtagatgatgaggatttcttgatgggtgaagatgtttacacaccaggaaaagagggagatgctttacgaagcatgtcaaacccagaacaatttggtcaaccatctcatatgaaagactatgtatacactgaaaaagataacggtggtgtgcatacgaattctggcattccaaataaagcagcttataacgtaattcaagcaatagggaaatctaaatcagaacaaatttactaccgagcattaacggaatacttaacaagtaattcaaacttcaaagattgtaaagatgcattataccaagcggctaaagatttatatgacgagcaaacagctgaacaagtatatgaagcatggaacgaagttggcgtcgagtaa

SEQ ID NO: 27 - DNA, 1548 bp, Staphylococcus aureus
  source 1..1548: mol_type = genomic DNA
atgaaaaagaaattaggtatgttacttcttgtaccagccgtaactttatcattagccgcatgtgggaatgatgatggaaaagataaagatggcaaggtaacaattaaaacgacagtttatccattgcaatcatttgcagagcaaattggtggaaaacacgtgaaggtatcatcaatctatccagcagggacagatttacatagctatgaaccaacacaaaaagatatattaagtgcaagcaagtcagacttgtttatgtatacaggggataatttagatccggttgctaagaaagttgcatctactattaaagataaagataaaaaactgtctttagaagataaattagataaagcaaagcttttaactgatcaacacgaacatggtgaagagcatgaacatgagggacatgatcatgggaaagaagaacatcatcatcatggcggatatgatccacacgtatggttagatcctaaaattaaccaaactttcgctaaagaaattaaagatgaattagtgaagaaagatccaaaacataaagatgactatgagaaaaactacaaaaaattaaacgacgatcttaagaaaattgataacgatatgaagcaagttactaaagataagcaaggtaatgcagtattcatttcacatgaatcaattggatacttagctgatcgttatggttttgttcaaaaaggtattcaaaacatgaatgctgaagatccatcacaaaaagaattgactaaaattgttaaagaaattagagatagcaatgctaaatatattctttacgaagataatgttgcgaataaagtgactgaaacaattcgtaaagaaacagatgcgaagcctttaaaattctacaacatggagtctttaaataaagaacaacagaaaaaagataatattacctatcaatcattaatgaaatcgaatattgaaaatatcggtaaagctttagacagtggtgttaaagtgaaagacgacaaagctgaaagtaaacacgacaaagcaatttctgatgggtattttaaagatgagcaagttaaagaccgtgaattaagcgattatgctggtgaatggcaatctgtttacccttacttaaaagacggtacgcttgatgaagtgatggaacataaagctgaaaatgatccgaagaaatctgctaaagatttaaaagcttattatgacaaaggatataaaactgatattactaacattgatataaaaggaaatgaaattacatttactaaagatggtacgaaacacactggtaaatatgaatacaatggtaagaaaacattgaaatatcctaaaggtaaccgtggcgtgagatttatgtttaaattggtcgatggtaatgataaagacttaccgaaattcatccaatttagcgatcacaacattgcacctaaaaaggcagaacacttccatatctttatgggtaatgataatgacgcgttattaaaagaaatggataactggccaacatattatccttcaaaattaaataaagaccaaatcaaagaagaaatgttagcgcattaa

SEQ ID NO: 28 - DNA, 1695 bp, Staphylococcus aureus
  source 1..1695: mol_type = genomic DNA
atggtgttatatatcattttggcaataattgtgattatattgattgctgtaggtgtattattctatttacgttcaaataaaagacaaataatagaaaaagcaatcgaacgtaaaaatgaaattgaaacgttaccttttgatcaaaaccttgcacaattatctaagttgaatttaaaaggtgaaacaaaaacgaaatacgatgcaatgaaaaaggacaacgtagaaagtacaaataagtatctagctcctgtggaagaaaaaatccataatgctgaggctttattagataaatttagtttcaacgcatctcaatgtgaaattgatgatgcaaatgagttgatggatagttacgaacaaagctatcagcaacaattagaagatgtaaatgaaattattgcgttatacaaagataatgatgaattatatgacaaatgtaaggttgattatcgtgaaatgaaacgtgatgttttagcaaatcgtcatcaatttggtgaggcagcaagtcttcttgaaactgaaattgaaaaattcgagccaaggttagagcaatatgaagtactaaaagctgatggtaattatgtacaagcgcacaaccatatagctgccttgaatgaacaaatgaaacagctaagatcttatatggaagaaataccagaattaattagagaaactcaaaaagaattacctggtcaattccaagatttaaaatatggttgccgtgatcttaaagttgaagggtatgatctggatcacgtaaaagtagacagtacattacaaagcttaaaaacagagcttagtttcgttgaaccattaattagtcgcttagaattagaagaagctaatgataaactagctaatatcaatgataagttagatgacatgtatgatttaattgaacatgaagttaaagctaaaaatgatgtcgaagaaacaaaagatatcattacggataacttattcaaagcaaaagacatgaattatacattgcaaacagaaattgaatatgtacgtgaaaactactatataaatgaatctgatgctcagagtgttcgtcaatttgaaaatgaaattcaaagtttaatttctgtatatgatgatattttaaaagaaatgtctaaatctgctgtacgatatagcgaggttcaggataatttacaatatttagaagatcatgtcacagttattaatgacaaacaagaaaagctacaaaatcatctgattcaattgcgtgaagatgaagcagaagcagaagacaatctgttacgagtacaatcgaagaaagaagaagtgtatcgtcgattacttgcttctaacttaacaagcgttcctgaaaggtttatcatcatgaaaaatgaaattgatcatgaagttcgtgatgttaacgaacaatttagtgaacgtccaatacacgttaaacagttaaaagataaagtgtctaaaattgtgattcaaatgaatacatttgaagatgaagcaaatgatgttcttgttaatgctgtttatgcagagaaattaattcaatatggaaatagatatcgtaaggactatagcaatgttgataagagcttaaatgaagctgaacgattatttaaaaataatcgctataagcgtgcgattgaaattgcagagcaagctcttgaaagtgttgagccaggtgtcactaaacatattgaagaagaagttattaagcaatag

SEQ ID NO: 29 - DNA, 1860 bp, Staphylococcus aureus
  source 1..1860: mol_type = genomic DNA
atgcctaaaaataaaattttaatttatttgctatcaactacgctcgtattacctactttagtttcacctaccgcttatgctgacacacctcaaaaagatactacagctaagacaacatctcatgattccaaaaaatctactgatgatgaaacttctaaggatactacaagtaaagatattgataaagcagacaacaataatactagtaaccaagacaataacgacaaaaaagttaaaactatagacgacagcacttcagactctaacaatatcattgattttatttataagaatttaccacaaaccaatataaaccaattgctaaccaaaaataaatacgatgataattactcattaacaactttaatccaaaacttattcaatttaaattcggatatttctgattacgaacaacctcgtaatggtgaaaagtcaacaaatgattcgaataaaaacagtgataatagcatcaaaaatgatacggatacgcaatcatctaaacaagataaagcagacaatcaaaaagcacctaaatcaaacaatacaaaaccaagtacatctaataagcaaccaaattcgccaaagccaacacaaccaaatcaatcaaatagtcaaccagcaagtgacgataaagtaaatcaaaaatcttcatcgaaagataatcaatcaatgtcagattcggctttagattctattttggatcaatacagtgaagatgcaaagaaaacacaaaaagattacgcatctcaatctaaaaaagacaaaaatgaaaaatctaatacaaagaatccacagttaccaacacaagatgaattgaaacataaatctaaacctgctcaatcattcaataacgatgttaatcaaaaggatacacgtgcaacatcactattcgaaacagatcctagtatatctaacaatgatgatagtggacaatttaacgttgttgactcaaaagatacacgtcaatttgtcaaatcaattgctaaagatgcacaccgcattggtcaagataacgatatttatgcgtctgtcatgattgcccaagcaatcttagaatctgactcaggtcgtagtgctttagctaagtcaccaaaccataatttattcggtatcaaaggtgcttttgaagggaattctgttccttttaacacattagaagctgatggtaatcaattgtatagtattaatgctggattccgaaaatatccaagcacgaaagaatcactaaaagattactctgaccttattaaaaatggtattgatggcaatcgaacaatttataaaccaacatggaaatcggaagccgattcttataaagatgcaacatcacacttatctaaaacatatgctacagatccaaactatgctaagaaattaaacagtattattaaacactatcaattaactcagtttgacgatgaacgtatgccagatttagataaatatgaacgttctatcaaggattatgatgattcatcagatgaattcaaacctttccgcgaggtatctgataatatgccatatccacatggccaatgtacttggtacgtatataaccgtatgaaacaatttggtacatctatctcaggtgatttaggtgatgcacataattggaataatcgagctcaataccgtgattatcaagtaagtcatacaccaaaacgtcatgctgctgttgtatttgaggctggacaatttggtgcagatcaacattacggtcatgtagcatttgttgaaaaagttaacagtgatggttctatcgttatttcagaatccaatgttaaaggattaggtatcatttctcatagaactatcaatgcagctgccgctgaagaattatcatatattacaggtaaataa

SEQ ID NO: 30 - DNA, 2046 bp, Staphylococcus aureus
  source 1..2046: mol_type = genomic DNA
atgatgaaaagtcaaaataagtatagtattcgtaaatttagtgtaggtgcatcttccattttaatagctacattactatttttaagtggtggacaagcacaagcagctgagaagcaagtgaatatgggaaattcacaggaggatacagttacagcacaatctattggggatcaacaaactagggaaaatgctaattatcaacgtgaaaacggtgttgacgaacagcaacatactgaaaatttaactaagaacttgcataatgataaaacaatatcagaagaaaatcatcgtaaaacagatgatttgaataaagatcaactaaaggatgataaaaaatcatcgcttaataataaaaatattcaacgtgatacaacaaaaaataacaatgctaatcctagggatgtaaatcaagggttagaacaggctattaatgatggcaaacaaagtaaagtggcgtcacagcaacagtcaaaagaggcagataatagtcaagacttaaacgctaataacaatctaccttcacaaagtcgaacaaaggtatcaccatcattaaataagtcagatcaaacaagtcaacgagaaattgttaatgagacagaaatagagaaagtacaaccgcaacaaaagaatcaagcgaatgataaaattactgaccacaattttaacaatgaacaagaagtgaaacctcaaaaagacgaaaaaacactatcagtttcagatttaaaaaacaatcaaaaatcaccagttgaaccaacaaaggacaatgacaagaaaaatggattaaatttattaaaaagtagtgcagtagcaacgttaccaaacaaagggacaaaggaacttactgcaaaagcgaaaggtgatcaaacgaataaagttgccaaacaagggcagtataaaaatcaagatcctatagttttagtgcatggtttcaatgggtttacagatgatattaatccttcagtgttagctcattattggggcggtaataaaatgaacattcgccaagatttagaagaaaatggttacaaagcttatgaagcaagtataagtgcttttggaagtaactatgaccgcgcagttgaactttattattatatcaaaggcggtcgtgtagattatggtgcagcacatgcagcaaaatatggacatgaacgttatggaaaaacatacgaaggaatttacaaagactggaaaccaggacagaaggtacaccttgttggacatagtatgggtggtcaaacgatacgtcaactagaagaattactgcgtaatggtagtcgtgaagaaatagagtatcaaaagaaacatagtggcgaaatttctccactattcaaaggtaataatgacaatatgatttcatcaattactactttaggaacgccacataatggaacgcatgcttcagatttagctggtaatgaagctttagtgagacaaattgtatttgatatcggtaaaatgtttggtaataaaaattcaagagtagacttcgggttggctcaatggggtctaaaacagaagccaaatgaatcatatattgattatgtcaaacgcgttaaacaatctaatttatggaaatcaaaagataatggattttacgatctgacgcgtgagggtgcaacagatttaaatcgtaaaacgtcgttgaaccctaacattgtgtataaaacatacactggtgaagcaacgcacaaagcattaaatagcgatagacaaaaagcagacttaaatatgtttttcccatttgtgattactggtaacttaatcggtaaagctactgaaaaagaatggcgagaaaacgatggtttagtatccgttatttcttctcaacatccatttaatcaagcttatacaaatgcgacggataaaattcaaaaaggcatttggcaagtaacgcctacaaaacatgattgggatcatgttgattttgtcggacaagatagttctgatacagtgcgcacaagagaagaattacaagatttttggcatcatttagcagacgatttagtgaaaactgaaaaggtgactgatactaagcaagcataa

SEQ ID NO: 31 - DNA, 2421 bp, Staphylococcus aureus
  source 1..2421: mol_type = genomic DNA
atgacaaataaaatgaagaaatggcaaaaattatccaccattacgttattaatgaccggagtgattgctttaaataatggtgaatttagaaatgttgataaacatcaaatcgctgtggctgatacgaatgttcaaacgccagattatgaaaaattgaagaagacgtggctcgacgttaactacggttatgatcagtatgatgagaataatcaagatatgaagaagaagtttgatgctaaagaaaaagaagccaagaagttacttgatgacatgaaaactgatacgaatagaacatatttgtggtcaggagctgaaaaccttgaaactaattcttctcacatgacaaaaacctatcgtaatatcgagaaaatcgcagaatcaatgcaacataagaatacggtattaaaaacagttgaaaacaagttgaaaataaaagaagccctagattggatgcacaaaaatgtttatggcaagaatccttctcaaaaagtcgaggatttaactaaaaatcgtaaggggcaaactacacccaagaataactcattgaattggtgggattatgaaattggtacgccaagagcattaacaaatacactacttctaatggatgatatgctcactaaagatgaaatgaaaaattattcaaaacctattagtacatatgcaccatccagtgacaaaattttatcttctgttggtgaatcagaagatgctaaaggtggaaatttagtggacatttctaaagtaaaacttttagaaagtgttattgaagaagatgtagatatgttgaaaaagtctatagattcttttaataaagtgttcacttatgttcaagattctgccactggtaaaggtcgcaatggattctataaagatggctcttacattgatcatcaagatgtcccttacactggtgcttatggtgttgtactattagagggtatttctcaaatgatgccgatgataaaagaatctccttttaaaactacacaagataatgctacattaagcaattggattgacgaagggtttatgccattaatctataaaggtgaaatgatggatttatcacgaggtagagctatcagtcgtgaaaatgaaacgagtcatacagcgtcagcgactgtaatgaaatcattgttgagattgaatgataccatggatgattcaacaaaaactagatataagcaaatcgttaaaacttctgttaattctgattcaagttacaaccaaaataattatttaaattcatattcagacatagctaaaatgaaaaagttaatgaatgatagtactatttctaaaaacgatttaacacagcaacttaaaatatataatgacatggatcgtgtcacctatcacaataaagacctggactttgcatttggtttaagtatgacatcgaaaaacatcgcacgatacgaaaatatcaacggagagaacttaaaaggttggcacaccggtgcaggcatgtcttatttatataacagcgatgtcaaacactatcgcgataacttctgggcaacagccgatatgacttgtcttccaggcactactactttaaatgatatgccatctactaatactaagaatgataaatcttttgttggcgggacaaaattaaataataaatacgcaagcatcggtatggattttgaaaatcaggacaaaactttaactgccaaaaaatcatatttcatattaaacgataaaattgtcttcttaggaactggcattaaaagtactgattcatcaaagaatccagttacaagtgttgaaaatcgcaaagcaaatgggtataaattatttaaagatgatattgaaattaccacttcagatgttaatgctcaggaaacccattcagtctttttagagtccaacgatactaaaaagaacattggttatcatttcttagacaagccaaaaataactgtaaaaaaagaaagtcatactggtaagtggagtgaaattaataaaagtcaaaaaaaagatgacaaaaaagatgagtattatgaagtaactcaaacacataatacatctgacagtaaatatgcatatgttttgtatcctggtttatcaaaaagtgattttaaatcgaagaataataatgtaagtattgttaaacaagatgaagattttcatgtgataaaagataatgatggcgtatttgctggggttaattatagtgataatactaaatcttttgatataaacggaattactgttgaattaaaagaaaaaggcatgtttgtaattaaaaagaaagatgataaagcatataaatgtagcttctataatcctgaaactacaaataccgcttcaaatatagaatcaaaaatttttattaaaggttacaccataactaataaaagtgtcataaactctaatgatgctggtgtaaactttgaattaactaaataa

SEQ ID NO: 32 - DNA, 2427 bp, Staphylococcus aureus
  source 1..2427: mol_type = genomic DNA
atgacatatagaatgaagaaatggcaaaaattgtccaccattacgttattaatggctggtgtgattactttgaatggtggtgaattcagaagtattgataaacatcaaatcgctgtggctgatacgaatgttcaaacgacagattatgaaaagttgaggaacatatggctggacgttaactatggttatgataagtatgatgagaataatccagatatgaagaagaagtttgaggctacggagaatgaggcagagaaattactcaaggaaatgaaaactgaaagtgataggaaatacttgtgggaaagctcaaaagatttagatacgaagtctgcggatatgactcgtacctatcgtaatattgagaaaatctcagaagcgatgaaacataaaaatactaaattaaaaacagatgaaaacaagacaaaagtaaaagatgcacttgagtggctgcataaaaatgcatatggaaaagaaccagataaaaaagttgctgatttgacctcaaactttaaaaataaaacttctagaaataccaacttaaattggtgggattatgaaattggaacacctagagcattaacaaatacgcttatactcttacaagaagatttcactgatgaagaaaagaaaaaatatacagctcctattaaaactttcgccccagatagtgacaaaatattatcttctgtaggaaaatctgaacctgctaaaggcggaaatttagtagacatttctaaagtaaaacttttagaaagtattatcgaagaagacaaagatatgatgaaaaagtctatagattcatttaatacagtcttcacttacgcgcaaaattctgccactggaaaagaacgtaatggattctataaagatggctcttacattgatcatcaagacgtcccatacactggtgcttatggcgttgtactattagagggtatttctcaaatgatgccgatgataaaagaaacaccttttaatgatagtaaccaaaatgatacaaccttaaaatcatggattgacgacggatttatgccactcatttataaaggtgaaatgatggatttatcaagaggtagagctatcagtcgtgaaaatgaaacgagtcactcagcatctgcaacagtaatgaaatcattgttgagattgagtgataccatggataagtctacaaaagctaaatataaaaagattgtcaagacttcagtagagtcagattcaagttataaacaaaccgattatttaagctcttattcggatataagcaaaatgaagtctttaatggaagacagcactatttctactaacggtttaacacaacaacttaaaatatataatgacatggatcgtgtcacctatcacaataaaggcttagactttgcatttggtttaagtatgacgtcgaaaaacgtcgcacgttacgaaagtatcaacggagagaacttaaaaggttggcacactggtgctggaatgtcttatttatacaatagcgatgtgaaacactaccgtgataacttctgggcgacagctgatatgaaacgtttagcaggtactacaactttagataatgaagaacctaaaagtacggatgttaaaaagtctagtaaaacttttgtaggaggaacaaaattcgatgaccaacatgctagtatcggaatggattttgaaaatcaggacaaaactttaactgccaaaaaatcatatttcatattaaacgataaaattgtcttcttaggaactggcattaaaagtactgattcatcaaagaatccagttacaacgattgaaaatcgcaaagcgaatgattataaattatataaagatgatacgcaaacaaccaattccgataatcaggaaaccaattccctctttttagagtcaacgaatagcactcaaaacaatataggttatcattttttaaacgaatcgaaaataactgtaaaaaaagaaagtcatactggtaagtggagtgatataaataaaagccaaaaggatatacaaaaaactgatgagtattatgaagtaactcaaaagcattctaatacagatagtaaatatgcatatgtgttgtatccaggcttatctaaagatgtctttaaatccaaagcaagcaaagtaactgtcgttaagcaagaagatgacttccacgttgtgaaagataatgaatcggtttgggctggtatcaattatagtgatagcgctaaaacttttgaaattaataacactaaagtcgaagttaaagccaaaggaatgtttattcttacaaagaaagatgataacacttatgaatgtagcttctataatcccgaatctacaaattccgtttcagatattgaatctaaaatttcaatgactggatactctattataaacaaaaatacgtcgacttctaatgaatccggcgtacgctttgaattaactaaataa

SEQ ID NO: 33 - RNA, 423 nt, Staphylococcus aureus
  source 1..423: mol_type = mRNA
atggcaaaaggtaatttatttaaagcgattttaggtataggtggcgctgtagcagctgtacttgttacacgtaaagatagtcgtgacaagctgaaagcagaatataataaatacaaacaagatcctcaaagctataaagataatgctaaggataaagcgacgcaattaggaacaattgcaaatgaaacaattaaagaagtaaaaacaaatccgaaagaatatgctaatagattaaaaaataatccaaaagcatttttcgaagaagaaaaatcaaaatttaccgaatatgacaataagactgacgaaagtattgaaaaaggtaaatttgatgatgaaggtggcgcagcaccaaataataatttacgtatcgtcactgaagaagatttaaaaaagaataaaaatgcattgtctgataaagaataa

SEQ ID NO: 34 - RNA, 582 nt, Staphylococcus aureus
  source 1..582: mol_type = mRNA
atgaaaaaattggtttcaattgttggcgcaacattattgttagctggatgtggatcacaaaatttagcaccattagaagaaaaaacaacagatttaagagaagataatcatcaactcaaactagatattcaagaacttaatcaacaaattagtgattctaaatctaaaattaaagggcttgaaaaggataaagaaaatagtaaaaaaactgcatctaataatacgaaaattaaattgatgaatgttacatcaacatactacgacaaagttgctaaagctttgaaatcctataacgatattgaaaaggatgtaagtaaaaacaaaggcgataagaatgttcaatcgaaattaaatcaaatttctaatgatattcaaagtgctcacacttcatacaaagatgctatcgatggtttatcacttagtgatgatgataaaaaaacgtctaaaaatatcgataaattaaactctgatttgaatcatgcatttgatgatattaaaaatggctatcaaaataaagataaaaaacaacttacaaaaggacaacaagcgttgtcaaaattaaacttaaatgcaaaatcatga

SEQ ID NO: 35 - RNA, 630 nt, Staphylococcus aureus
  source 1..630: mol_type = mRNA
atgaaaaaattagttacagggttattagcattatcattatttttagctgcatgtggtcaagatagtgaccaacaaaaagacagtaataaagaaaaagatgataaagcgaaaactgaacaacaagataaaaaaacaaatgattcatctaaagataagaaagacaataaagatgatagtaaagacgtaaacaaagataataaagataatagtgcaaacgataaccagcaacaatctaattcaaatgcaacaaacaatgaccaaaatcaaacgaataataaccagtcaaacagtggacaaacgactaacaatcaaaaatcaagttacgttgcaccatattatggacaaaacgcagcgccagtggctcgtcaaatttatccatttaatggtaataaatcacaagcattacaacaattgcctaatttccaaacagctttaaatgcagctaacaacgaagcaaataaatttggtaatggtcataaagtttataatgattattcaattgaagaacataatggtaactataagtatgtttttagttttaaagacccaaacgtaaatggaaaatattcaattgtaacggttgattatactggacaagcaatggttactgatccaaactaccaacaataa

SEQ ID NO: 36 - RNA, 729 nt, Staphylococcus aureus
  source 1..729: mol_type = mRNA
atgaaaaaagtaatggggatattattagcaagtacacttatcttaggtgcttgtggacatcatcaagatagtgcaaaaaaagagagcactagtcacaaaaagaaagaaaatgacaatgaagaattaaatgaagaacttaaagaatttaaaagcaaaaaaaatatggatataaaaattaaaggcgatactattgttagtgacaaatttgaagctaaaataaaagaaccgtttatcatcaatgaaaaagatgagaaaaagaaatatatcgcttttaaaatggaaattactgctaaaaaagacgataaagatttaaatccatcttctatttctcatgactatattaatatcactcaagatgataaaaatacagtaaataaattaagagatggttatcttttaagtgataaaaattataaagattggacagaacataaccaagatcaaattaaaaaaggcaaaactgcacaagccatgtttatctatgagttaagaggtgatggaaacattaatttaaatgtccataaatactcagaagataaaacagttgattctaaatcattcaaatttagtaaacttaaaaccgaagatttttctcatagagcggaaacaagggaagaagtagaaaagaaagaaaaagaatttgaagaagagtacaaaaaagaacaagaacgagagaaagaaaaagaaaagcaaaaagatgacgaccacagtggtttagatgaagtataa

SEQ ID NO: 37 - RNA, 984 nt, Staphylococcus aureus
  source 1..984: mol_type = mRNA
atgaaaaaatggcaatttgttggtactacagctttaggtgcaacactattattaggtgcttgtggtggcggtaatggtggcagtggtaatagtgatttaaaaggggaagctaaaggggatggctcatcaacagtagcaccaattgtggagaaattaaatgaaaaatgggctcaagatcactcggatgctaaaatctcagcaggacaagctggtacaggtgctggtttccaaaaattcattgcaggagatatcgacttcgctgatgcttctagaccaattaaagatgaagagaagcaaaaattacaagataagaatatcaaatacaaagaattcaaaattgcgcaagatggtgtaacggttgctgtaaataaagaaaatgattttgtagatgaattagacaaacagcaattaaaagcaatttattctggaaaagctaaaacatggaaagatgttaatagtaaatggccagataaaaaaataaatgctgtatcaccaaactcaagtcatggtacttatgacttctttgaaaatgaagtaatgaataaagaagatattaaagcagaaaaaaatgctgatacaaatgctatcgtttcttctgtaacgaaaaacaaagagggaatcggatactttggatataacttctacgtacaaaataaagataaattaaaagaagttaaaatcaaagatgaaaatggtaaagcaacagagcctacgaaaaaaacaattcaagataactcttatgcattaagtagaccattattcatttatgtaaatgaaaaagcattgaaagataataaagtaatgtcagaatttatcaaattcgtcttagaagataaaggtaaagcagctgaagaaggtggatatgtagcagcaccagagaaaacatacaaatcacaattagatgatttaaaagcatttattgataaaaatcaaaaatcagacgacaagaaatctgatgataaaaagtctgaagacaagaaataa

SEQ ID NO: 38 - RNA, 1074 nt, Staphylococcus aureus
  source 1..1074: mol_type = mRNA
atgaaaggtaaatttttaaaagttagttctttattcgttgcaactttgacaacagcgacacttgtgagttctccagcagcaaatgcgttatcttcaaaagctatggacaatcatccacaacaaacgcagacagacaaacagcaaacacctaagattcaaaaaggcggtaaccttaaaccattagaacaacgtgaacgcgctaatgttatattaccaaataacgatcgtcaccaaatcacagatacaacgaatggtcattatgcacctgttacttatattcaagttgaagcacctactggtacatttattgcttctggtgtagttgtaggtaaagatacacttttaacaaataaacacatcgtagatgctacgcacggtgatcctcatgctttaaaagcattcgcttctgcaattaaccaagacaattatcctaatggtggtttcactgctgaacaaatcactaaatattcaggcgaaggtgatttagcaatcgttaaattctcccctaatgagcaaaacaaacatattggcgaagtagttaaaccagcaacaatgagtaataatgctgaaacacaagttaaccaaaatattactgtaacaggatatcctggtgataaacctgtcgcaacaatgtgggaaagtaaaggaaaaataacgtacttaaaaggtgaagcaatgcaatatgatttaagtacaactggtggtaactcaggttcacctgtatttaatgaaaaaaatgaagtcattggcattcattggggtggcgttccaaatcaatttaacggtgcagtatttattaatgaaaatgtacgcaacttcttaaaacaaaatattgaagatatcaatttcgcaaatgatgaccaccctaacaaccctgataatccagacaatccaaataatccggacaatcctaacaaccctgataaccctaacaaccctgataatccagacaatcctaataatcctgataaccctaacaacccggacaatccaaataaccctgaccaacctaacaacccaaataacccggacaatggcgataacaataattcagacaaccctgacgctgcataa

SEQ ID NO: 39 - RNA, 1200 nt, Staphylococcus aureus
  source 1..1200: mol_type = mRNA
atgaagcgtacattagtattattgattacagctatctttatactcgctgcttgtggtaaccataaggatgaccaggctggaaaagataatcaaaaacataacaatagttcaaatcaagtaaaagaaattgctacggataaaaatgtacaaggtgataactatcgtacattgttaccatttaaagaaagccaggcaagaggacttttacaagataacatggcaaatagttataatggcggcgactttgaagatggtttattgaacttaagtaaagaagtgtttccaacagacaaatatttgtatcaagatggtcaatttttggacaagaaaacaattaatgcctatttaaatcttaagtatacaaaacgtgaaatcgataaaatgtctgaaaaagataaaaaagacaagaaagcgaatgaaaatttaggacttaatccatcacacgaaggtgaaacagatcctgaaaagattgcagaaaaatcaccagcctatttatctaacattttagagcaagatttttatggtggtggagatacaaaaggtaagaatattaaaggtatgacgattggtttagctatgaatagtgtttattactataaaaaagaaaaagatggaccgacttttagtaaaaaactagatgatagcgaagttaaaaagcaaggtaaacaaatggctagtgagatattatcaaggttacgtgaaaatgatgatttaaaagatataccaattcattttgcaatttataagcaatcaagtgaagattcaatcacaccaggtgaatttatcactcaagcgactgcagaaaagagtcaaacaaagcttaatgaatggcataatatcaatgaaaaatcagctttattaccttcttcaacagcagcagattatgatgaaaatttaaataataatttcaagcaatttaatgataatttgcaatcatatttttctaatttcacacaagcagtaggaaaagttaaatttgttgataaaaagccacaacgattagtagtagatttaccaatcgattactatggacaagctgaaacaattggtattacacagtacgttactgaacaagcgaataaatatttcgataaaatcgataactatgaaattcggattaaagatggtaaccaaccacgtgctttaattagtaagacaaaagatgacaaagaaccgcaagttcatatttacagtaattaa

SEQ ID NO: 40 - RNA, 1488 nt, Staphylococcus aureus
  source 1..1488: mol_type = mRNA
atgagggaaaattttaagttacgtaaaatgaaagtcgggttagtatctgttgcaattacaatgttatatatcatgacaaacggacaagcagaagcatcagaggctaatgagaagccaagtacaaatcaagaatcaaaagttgtttcacagactgaacaaaattcaaaagaaacaaaaacagtagaatctaataagaactttgttaaattagatactattaaacctggagctcaaaagataacgggaactactttaccaaatcactatgttttattaacagttgatgggaaaagtgcggattcagtagaaaatggcggtttgggttttgttgaagcaaatgacaaaggagaatttgagtaccctttaaataatcgtaaaattgttcataatcaagaaattgaggtttcgtcgtcaagccctgatttaggtgaagatgaagaagatgaagaggtggaagaagcttcaactgataaagctggcgttgaggaagaaagtacagaagctaaagttacttacacaacaccgcgatatgaaaaagcgtatgaaataccgaaagaacaactaaaagaaaaagatggacatcaccaagtttttatcgaacctattactgaaggatcaggtattattaaagggcatacgtctgtaaaaggtaaagttgctttatctattaataataaatttattaattttgaagagagcgttaagggcggagttagtaaagaagacactaaagctagttcagatggtatctggatgcctattgatgacaaaggatactttaactttgacttcaaaacgaaacgtttcgataatttagagttaaaagaaggtaatgacatttcactaacatttgcacctgatgatgaagaagatgcattaaaacctttaattttcaaaactaaagtaacgagcttagaagatatcgataaagcagaaactaaatatgaccatactaaactcaacaaagtgaaagttttagataatgttaaagaagatttacatgttgatgaaatatatggaagcttatatcatacagacaaaggtaaaggtattcttgataaagaaggtactaaagtaattaaaggaaagactaaattcgcgaatgcagtagtgaaggtagactctgaactaggtgaagcacaattattccctgatttacaagtaaatgaaaaaggtgaatttagctttgactcacatggtgctggttttagattacaaaatggagaaaaattaaacttcacagtggttgatcctattacaggtgacttgttaagtaatgagtttgtttctaaagagattgatattgaagaaacacctgaacaaaaagcggatcgtgagtttgacgaaaaacttgaaaatacgcctgcttactacaagttatacggcgataaaatagttggattcgatactaacgatttcccgattacttggttctatccattgggtgaaaagaaagttgaacgtacaacacctaaattagaaaaataa

SEQ ID NO: 41 - RNA, 1524 nt, Staphylococcus aureus
  source 1..1524: mol_type = mRNA
atgtctaaaaagttaaaaattataattcctattattattgtcttattattaataggtggaatcgcatggggagtttatgcattttttgcaaacacaccgaaaaatacatacttaaaaagtgaacaacaaactgcaaaaatgtataaagattattttaatgaccgttttgaaaacgaagtgaagttccaagaaaagatgaaagataattcatttttatcttcattagaattaagcgcagatgcatctgatgaaattgttaaagggcttggtattcctaaatctgttgttaatgcttcgaaaattaaaatgtcatatggacatgatcctaaaaaagagaaatcaatgattaatcttgaaccaacaatagcagactctgcattagggaaattccagttagctgcagataaagataagcattatttcgaatcaccattatttaaagggaaatatagtgttaataattctgatttattatcaacttattcaaaacttacaggtgaagatgaagaaacagcaaaagaaaatggtattacaaaccaacaactaaatttaaatactcttttcagtaatgctcaagcacaacaaagtgactacagcaaaattgccgaaaaatattccgaacttattgtcgacaaattagatgacgataattttgataaaggtaaaaaagaagaaattaaggttaatggtgaaaagtacaaagttagacctgtcacgttaacacttagcagagctgacactaaaaaaattacattagctgtattagaagaagctaaaaaggataaagaccttaaaaaattaatggaagaacaaggtactacaaaagactttgaaaaagacattaaaaaagcaattgacgatgtcaaagaaactaaaaaggatgaatttgctaaaattcaatctaaaatttataccgaaaaacatacgattgtaaaacgagaaattactattacagacaaagaaaataataaaactaaaatcaaaggtactaatactttagaagacgataagttaaaactagattacgcacttgatttcgatcaagataaatacacgtatgctgaagcgaaatatacaattaaaggcgtatcttctaaggaaaaagacaataaatacagtgataaatacgaatttggtaaaaagacagaatatgatgaatcaaaaatcaaattagataaccaagaaaaagtagatggcacaaaacgtcaagataaaggtaaaatcactgtcgcgttagataaatatagcgacgaaaatgaattcacttttgaaaataatatagattctgacgtaaaaaataacactcagaaatctacgttaaatatcggcatcaaatatgctgaagaaccaattaatttcattttaaaatctagcacaaaattgaaagcagatattgattttgatgatagtggtgcgaaagatttcaatagtctatcttcaaaagaccgtgaaaaacttgaaaaagaaatcgaaaaaaatggcggcaaaatgtttgaatcaattttaaaaaaggcatctaaataa

SEQ ID NO: 42 - RNA, 1530 nt, Staphylococcus aureus
  source 1..1530: mol_type = mRNA
gtgaggaaattttcaagatatgcatttacaagtatggcaacagtaacgttgctgagctctttgacacctgcagcactagcgagtgatacgaatcacaaaccagcaacttcagatattaattttgaaatcacgcaaaagagtgatgcagttaaagcattaaaagagttacctaaatctgaaaatgtgaaaaatcattatcaagattactctgttacagatgtaaaaacagataagaaaggattcacgcattacacgttacaaccgagtgtggatggtgtgcatgcgcctgacaaagaagtgaaagtgcatgcggacaaatcgggtaaagtcgttttaatcaacggtgatactgatgcgaagaaagtaaagccgacaaataaagtgacattaagcaaggatgaagcggctgacaaagcatttaacgcagttaagattgataaaaataaagctaaaaacctccaagatgacgttatcaaagaaaataaagtcgaaatcgatggtgacagtaataaatacatttacaatattgaattaattacagtaacaccagaaatttcacattggaaagttaaaattgatgcagacacaggagcagttgttgaaaaaacgaacttagttaaagaagcagcagcaactggcacaggtaaaggtgtgcttggagatacaaaagatatcaatatcaatagtattgatggtggatttagtttagaggatttgacgcatcaaggtaaattatcagcatacaattttaacgatcaaacaggtcaagcgacattaattactaatgaagatgaaaacttcgtcaaagatgatcaacgtgctggtgtagatgcgaattattatgctaaacaaacatatgattactacaaaaatacatttggtcgtgagtcttacgataaccatggtagtccaatagtctcattaacacatgtaaatcattatggtggacaagataacagaaataacgctgcatggattggagacaaaatgatttatggtgatggcgatggccgcacgtttacaaatttatcaggtgcaaatgacgtagtagcacatgagttaacacatggcgtgacacaagaaacggcgaatttagagtataaagatcaatctggtgcgttaaatgaaagcttttcagatgtttttggatactttgtagatgatgaggatttcttgatgggtgaagatgtttacacaccaggaaaagagggagatgctttacgaagcatgtcaaacccagaacaatttggtcaaccatctcatatgaaagactatgtatacactgaaaaagataacggtggtgtgcatacgaattctggcattccaaataaagcagcttataacgtaattcaagcaatagggaaatctaaatcagaacaaatttactaccgagcattaacggaatacttaacaagtaattcaaacttcaaagattgtaaagatgcattataccaagcggctaaagatttatatgacgagcaaacagctgaacaagtatatgaagcatggaacgaagttggcgtcgagtaa

SEQ ID NO: 43 - RNA, 1548 nt, Staphylococcus aureus
  source 1..1548: mol_type = mRNA
atgaaaaagaaattaggtatgttacttcttgtaccagccgtaactttatcattagccgcatgtgggaatgatgatggaaaagataaagatggcaaggtaacaattaaaacgacagtttatccattgcaatcatttgcagagcaaattggtggaaaacacgtgaaggtatcatcaatctatccagcagggacagatttacatagctatgaaccaacacaaaaagatatattaagtgcaagcaagtcagacttgtttatgtatacaggggataatttagatccggttgctaagaaagttgcatctactattaaagataaagataaaaaactgtctttagaagataaattagataaagcaaagcttttaactgatcaacacgaacatggtgaagagcatgaacatgagggacatgatcatgggaaagaagaacatcatcatcatggcggatatgatccacacgtatggttagatcctaaaattaaccaaactttcgctaaagaaattaaagatgaattagtgaagaaagatccaaaacataaagatgactatgagaaaaactacaaaaaattaaacgacgatcttaagaaaattgataacgatatgaagcaagttactaaagataagcaaggtaatgcagtattcatttcacatgaatcaattggatacttagctgatcgttatggttttgttcaaaaaggtattcaaaacatgaatgctgaagatccatcacaaaaagaattgactaaaattgttaaagaaattagagatagcaatgctaaatatattctttacgaagataatgttgcgaataaagtgactgaaacaattcgtaaagaaacagatgcgaagcctttaaaattctacaacatggagtctttaaataaagaacaacagaaaaaagataatattacctatcaatcattaatgaaatcgaatattgaaaatatcggtaaagctttagacagtggtgttaaagtgaaagacgacaaagctgaaagtaaacacgacaaagcaatttctgatgggtattttaaagatgagcaagttaaagaccgtgaattaagcgattatgctggtgaatggcaatctgtttacccttacttaaaagacggtacgcttgatgaagtgatggaacataaagctgaaaatgatccgaagaaatctgctaaagatttaaaagcttattatgacaaaggatataaaactgatattactaacattgatataaaaggaaatgaaattacatttactaaagatggtacgaaacacactggtaaatatgaatacaatggtaagaaaacattgaaatatcctaaaggtaaccgtggcgtgagatttatgtttaaattggtcgatggtaatgataaagacttaccgaaattcatccaatttagcgatcacaacattgcacctaaaaaggcagaacacttccatatctttatgggtaatgataatgacgcgttattaaaagaaatggataactggccaacatattatccttcaaaattaaataaagaccaaatcaaagaagaaatgttagcgcattaa

SEQ ID NO: 44 - RNA, 1695 nt, Staphylococcus aureus
  source 1..1695: mol_type = mRNA
atggtgttatatatcattttggcaataattgtgattatattgattgctgtaggtgtattattctatttacgttcaaataaaagacaaataatagaaaaagcaatcgaacgtaaaaatgaaattgaaacgttaccttttgatcaaaaccttgcacaattatctaagttgaatttaaaaggtgaaacaaaaacgaaatacgatgcaatgaaaaaggacaacgtagaaagtacaaataagtatctagctcctgtggaagaaaaaatccataatgctgaggctttattagataaatttagtttcaacgcatctcaatgtgaaattgatgatgcaaatgagttgatggatagttacgaacaaagctatcagcaacaattagaagatgtaaatgaaattattgcgttatacaaagataatgatgaattatatgacaaatgtaaggttgattatcgtgaaatgaaacgtgatgttttagcaaatcgtcatcaatttggtgaggcagcaagtcttcttgaaactgaaattgaaaaattcgagccaaggttagagcaatatgaagtactaaaagctgatggtaattatgtacaagcgcacaaccatatagctgccttgaatgaacaaatgaaacagctaagatcttatatggaagaaataccagaattaattagagaaactcaaaaagaattacctggtcaattccaagatttaaaatatggttgccgtgatcttaaagttgaagggtatgatctggatcacgtaaaagtagacagtacattacaaagcttaaaaacagagcttagtttcgttgaaccattaattagtcgcttagaattagaagaagctaatgataaactagctaatatcaatgataagttagatgacatgtatgatttaattgaacatgaagttaaagctaaaaatgatgtcgaagaaacaaaagatatcattacggataacttattcaaagcaaaagacatgaattatacattgcaaacagaaattgaatatgtacgtgaaaactactatataaatgaatctgatgctcagagtgttcgtcaatttgaaaatgaaattcaaagtttaatttctgtatatgatgatattttaaaagaaatgtctaaatctgctgtacgatatagcgaggttcaggataatttacaatatttagaagatcatgtcacagttattaatgacaaacaagaaaagctacaaaatcatctgattcaattgcgtgaagatgaagcagaagcagaagacaatctgttacgagtacaatcgaagaaagaagaagtgtatcgtcgattacttgcttctaacttaacaagcgttcctgaaaggtttatcatcatgaaaaatgaaattgatcatgaagttcgtgatgttaacgaacaatttagtgaacgtccaatacacgttaaacagttaaaagataaagtgtctaaaattgtgattcaaatgaatacatttgaagatgaagcaaatgatgttcttgttaatgctgtttatgcagagaaattaattcaatatggaaatagatatcgtaaggactatagcaatgttgataagagcttaaatgaagctgaacgattatttaaaaataatcgctataagcgtgcgattgaaattgcagagcaagctcttgaaagtgttgagccaggtgtcactaaacatattgaagaagaagttattaagcaatag

SEQ ID NO: 45 - RNA, 1860 nt, Staphylococcus aureus
  source 1..1860: mol_type = mRNA
atgcctaaaaataaaattttaatttatttgctatcaactacgctcgtattacctactttagtttcacctaccgcttatgctgacacacctcaaaaagatactacagctaagacaacatctcatgattccaaaaaatctactgatgatgaaacttctaaggatactacaagtaaagatattgataaagcagacaacaataatactagtaaccaagacaataacgacaaaaaagttaaaactatagacgacagcacttcagactctaacaatatcattgattttatttataagaatttaccacaaaccaatataaaccaattgctaaccaaaaataaatacgatgataattactcattaacaactttaatccaaaacttattcaatttaaattcggatatttctgattacgaacaacctcgtaatggtgaaaagtcaacaaatgattcgaataaaaacagtgataatagcatcaaaaatgatacggatacgcaatcatctaaacaagataaagcagacaatcaaaaagcacctaaatcaaacaatacaaaaccaagtacatctaataagcaaccaaattcgccaaagccaacacaaccaaatcaatcaaatagtcaaccagcaagtgacgataaagtaaatcaaaaatcttcatcgaaagataatcaatcaatgtcagattcggctttagattctattttggatcaatacagtgaagatgcaaagaaaacacaaaaagattacgcatctcaatctaaaaaagacaaaaatgaaaaatctaatacaaagaatccacagttaccaacacaagatgaattgaaacataaatctaaacctgctcaatcattcaataacgatgttaatcaaaaggatacacgtgcaacatcactattcgaaacagatcctagtatatctaacaatgatgatagtggacaatttaacgttgttgactcaaaagatacacgtcaatttgtcaaatcaattgctaaagatgcacaccgcattggtcaagataacgatatttatgcgtctgtcatgattgcccaagcaatcttagaatctgactcaggtcgtagtgctttagctaagtcaccaaaccataatttattcggtatcaaaggtgcttttgaagggaattctgttccttttaacacattagaagctgatggtaatcaattgtatagtattaatgctggattccgaaaatatccaagcacgaaagaatcactaaaagattactctgaccttattaaaaatggtattgatggcaatcgaacaatttataaaccaacatggaaatcggaagccgattcttataaagatgcaacatcacacttatctaaaacatatgctacagatccaaactatgctaagaaattaaacagtattattaaacactatcaattaactcagtttgacgatgaacgtatgccagatttagataaatatgaacgttctatcaaggattatgatgattcatcagatgaattcaaacctttccgcgaggtatctgataatatgccatatccacatggccaatgtacttggtacgtatataaccgtatgaaacaatttggtacatctatctcaggtgatttaggtgatgcacataattggaataatcgagctcaataccgtgattatcaagtaagtcatacaccaaaacgtcatgctgctgttgtatttgaggctggacaatttggtgcagatcaacattacggtcatgtagcatttgttgaaaaagttaacagtgatggttctatcgttatttcagaatccaatgttaaaggattaggtatcatttctcatagaactatcaatgcagctgccgctgaagaattatcatatattacaggtaaataa

SEQ ID NO: 46 - RNA, 2046 nt, Staphylococcus aureus
  source 1..2046: mol_type = mRNA
atgatgaaaagtcaaaataagtatagtattcgtaaatttagtgtaggtgcatcttccattttaatagctacattactatttttaagtggtggacaagcacaagcagctgagaagcaagtgaatatgggaaattcacaggaggatacagttacagcacaatctattggggatcaacaaactagggaaaatgctaattatcaacgtgaaaacggtgttgacgaacagcaacatactgaaaatttaactaagaacttgcataatgataaaacaatatcagaagaaaatcatcgtaaaacagatgatttgaataaagatcaactaaaggatgataaaaaatcatcgcttaataataaaaatattcaacgtgatacaacaaaaaataacaatgctaatcctagggatgtaaatcaagggttagaacaggctattaatgatggcaaacaaagtaaagtggcgtcacagcaacagtcaaaagaggcagataatagtcaagacttaaacgctaataacaatctaccttcacaaagtcgaacaaaggtatcaccatcattaaataagtcagatcaaacaagtcaacgagaaattgttaatgagacagaaatagagaaagtacaaccgcaacaaaagaatcaagcgaatgataaaattactgaccacaattttaacaatgaacaagaagtgaaacctcaaaaagacgaaaaaacactatcagtttcagatttaaaaaacaatcaaaaatcaccagttgaaccaacaaaggacaatgacaagaaaaatggattaaatttattaaaaagtagtgcagtagcaacgttaccaaacaaagggacaaaggaacttactgcaaaagcgaaaggtgatcaaacgaataaagttgccaaacaagggcagtataaaaatcaagatcctatagttttagtgcatggtttcaatgggtttacagatgatattaatccttcagtgttagctcattattggggcggtaataaaatgaacattcgccaagatttagaagaaaatggttacaaagcttatgaagcaagtataagtgcttttggaagtaactatgaccgcgcagttgaactttattattatatcaaaggcggtcgtgtagattatggtgcagcacatgcagcaaaatatggacatgaacgttatggaaaaacatacgaaggaatttacaaagactggaaaccaggacagaaggtacaccttgttggacatagtatgggtggtcaaacgatacgtcaactagaagaattactgcgtaatggtagtcgtgaagaaatagagtatcaaaagaaacatagtggcgaaatttctccactattcaaaggtaataatgacaatatgatttcatcaattactactttaggaacgccacataatggaacgcatgcttcagatttagctggtaatgaagctttagtgagacaaattgtatttgatatcggtaaaatgtttggtaataaaaattcaagagtagacttcgggttggctcaatggggtctaaaacagaagccaaatgaatcatatattgattatgtcaaacgcgttaaacaatctaatttatggaaatcaaaagataatggattttacgatctgacgcgtgagggtgcaacagatttaaatcgtaaaacgtcgttgaaccctaacattgtgtataaaacatacactggtgaagcaacgcacaaagcattaaatagcgatagacaaaaagcagacttaaatatgtttttcccatttgtgattactggtaacttaatcggtaaagctactgaaaaagaatggcgagaaaacgatggtttagtatccgttatttcttctcaacatccatttaatcaagcttatacaaatgcgacggataaaattcaaaaaggcatttggcaagtaacgcctacaaaacatgattgggatcatgttgattttgtcggacaagatagttctgatacagtgcgcacaagagaagaattacaagatttttggcatcatttagcagacgatttagtgaaaactgaaaaggtgactgatactaagcaagcataa

SEQ ID NO: 47 - RNA, 2421 nt, Staphylococcus aureus
  source 1..2421: mol_type = mRNA
atgacaaataaaatgaagaaatggcaaaaattatccaccattacgttattaatgaccggagtgattgctttaaataatggtgaatttagaaatgttgataaacatcaaatcgctgtggctgatacgaatgttcaaacgccagattatgaaaaattgaagaagacgtggctcgacgttaactacggttatgatcagtatgatgagaataatcaagatatgaagaagaagtttgatgctaaagaaaaagaagccaagaagttacttgatgacatgaaaactgatacgaatagaacatatttgtggtcaggagctgaaaaccttgaaactaattcttctcacatgacaaaaacctatcgtaatatcgagaaaatcgcagaatcaatgcaacataagaatacggtattaaaaacagttgaaaacaagttgaaaataaaagaagccctagattggatgcacaaaaatgtttatggcaagaatccttctcaaaaagtcgaggatttaactaaaaatcgtaaggggcaaactacacccaagaataactcattgaattggtgggattatgaaattggtacgccaagagcattaacaaatacactacttctaatggatgatatgctcactaaagatgaaatgaaaaattattcaaaacctattagtacatatgcaccatccagtgacaaaattttatcttctgttggtgaatcagaagatgctaaaggtggaaatttagtggacatttctaaagtaaaacttttagaaagtgttattgaagaagatgtagatatgttgaaaaagtctatagattcttttaataaagtgttcacttatgttcaagattctgccactggtaaaggtcgcaatggattctataaagatggctcttacattgatcatcaagatgtcccttacactggtgcttatggtgttgtactattagagggtatttctcaaatgatgccgatgataaaagaatctccttttaaaactacacaagataatgctacattaagcaattggattgacgaagggtttatgccattaatctataaaggtgaaatgatggatttatcacgaggtagagctatcagtcgtgaaaatgaaacgagtcatacagcgtcagcgactgtaatgaaatcattgttgagattgaatgataccatggatgattcaacaaaaactagatataagcaaatcgttaaaacttctgttaattctgattcaagttacaaccaaaataattatttaaattcatattcagacatagctaaaatgaaaaagttaatgaatgatagtactatttctaaaaacgatttaacacagcaacttaaaatatataatgacatggatcgtgtcacctatcacaataaagacctggactttgcatttggtttaagtatgacatcgaaaaacatcgcacgatacgaaaatatcaacggagagaacttaaaaggttggcacaccggtgcaggcatgtcttatttatataacagcgatgtcaaacactatcgcgataacttctgggcaacagccgatatgacttgtcttccaggcactactactttaaatgatatgccatctactaatactaagaatgataaatcttttgttggcgggacaaaattaaataataaatacgcaagcatcggtatggattttgaaaatcaggacaaaactttaactgccaaaaaatcatatttcatattaaacgataaaattgtcttcttaggaactggcattaaaagtactgattcatcaaagaatccagttacaagtgttgaaaatcgcaaagcaaatgggtataaattatttaaagatgatattgaaattaccacttcagatgttaatgctcaggaaacccattcagtctttttagagtccaacgatactaaaaagaacattggttatcatttcttagacaagccaaaaataactgtaaaaaaagaaagtcatactggtaagtggagtgaaattaataaaagtcaaaaaaaagatgacaaaaaagatgagtattatgaagtaactcaaacacataatacatctgacagtaaatatgcatatgttttgtatcctggtttatcaaaaagtgattttaaatcgaagaataataatgtaagtattgttaaacaagatgaagattttcatgtgataaaagataatgatggcgtatttgctggggttaattatagtgataatactaaatcttttgatataaacggaattactgttgaattaaaagaaaaaggcatgtttgtaattaaaaagaaagatgataaagcatataaatgtagcttctataatcctgaaactacaaataccgcttcaaatatagaatcaaaaatttttattaaaggttacaccataactaataaaagtgtcataaactctaatgatgctggtgtaaactttgaattaactaaataa

SEQ ID NO: 48 - RNA, 2427 nt, Staphylococcus aureus
  source 1..2427: mol_type = mRNA
atgacatatagaatgaagaaatggcaaaaattgtccaccattacgttattaatggctggtgtgattactttgaatggtggtgaattcagaagtattgataaacatcaaatcgctgtggctgatacgaatgttcaaacgacagattatgaaaagttgaggaacatatggctggacgttaactatggttatgataagtatgatgagaataatccagatatgaagaagaagtttgaggctacggagaatgaggcagagaaattactcaaggaaatgaaaactgaaagtgataggaaatacttgtgggaaagctcaaaagatttagatacgaagtctgcggatatgactcgtacctatcgtaatattgagaaaatctcagaagcgatgaaacataaaaatactaaattaaaaacagatgaaaacaagacaaaagtaaaagatgcacttgagtggctgcataaaaatgcatatggaaaagaaccagataaaaaagttgctgatttgacctcaaactttaaaaataaaacttctagaaataccaacttaaattggtgggattatgaaattggaacacctagagcattaacaaatacgcttatactcttacaagaagatttcactgatgaagaaaagaaaaaatatacagctcctattaaaactttcgccccagatagtgacaaaatattatcttctgtaggaaaatctgaacctgctaaaggcggaaatttagtagacatttctaaagtaaaacttttagaaagtattatcgaagaagacaaagatatgatgaaaaagtctatagattcatttaatacagtcttcacttacgcgcaaaattctgccactggaaaagaacgtaatggattctataaagatggctcttacattgatcatcaagacgtcccatacactggtgcttatggcgttgtactattagagggtatttctcaaatgatgccgatgataaaagaaacaccttttaatgatagtaaccaaaatgatacaaccttaaaatcatggattgacgacggatttatgccactcatttataaaggtgaaatgatggatttatcaagaggtagagctatcagtcgtgaaaatgaaacgagtcactcagcatctgcaacagtaatgaaatcattgttgagattgagtgataccatggataagtctacaaaagctaaatataaaaagattgtcaagacttcagtagagtcagattcaagttataaacaaaccgattatttaagctcttattcggatataagcaaaatgaagtctttaatggaagacagcactatttctactaacggtttaacacaacaacttaaaatatataatgacatggatcgtgtcacctatcacaataaaggcttagactttgcatttggtttaagtatgacgtcgaaaaacgtcgcacgttacgaaagtatcaacggagagaacttaaaaggttggcacactggtgctggaatgtcttatttatacaatagcgatgtgaaacactaccgtgataacttctgggcgacagctgatatgaaacgtttagcaggtactacaactttagataatgaagaacctaaaagtacggatgttaaaaagtctagtaaaacttttgtaggaggaacaaaattcgatgaccaacatgctagtatcggaatggattttgaaaatcaggacaaaactttaactgccaaaaaatcatatttcatattaaacgataaaattgtcttcttaggaactggcattaaaagtactgattcatcaaagaatccagttacaacgattgaaaatcgcaaagcgaatgattataaattatataaagatgatacgcaaacaaccaattccgataatcaggaaaccaattccctctttttagagtcaacgaatagcactcaaaacaatataggttatcattttttaaacgaatcgaaaataactgtaaaaaaagaaagtcatactggtaagtggagtgatataaataaaagccaaaaggatatacaaaaaactgatgagtattatgaagtaactcaaaagcattctaatacagatagtaaatatgcatatgtgttgtatccaggcttatctaaagatgtctttaaatccaaagcaagcaaagtaactgtcgttaagcaagaagatgacttccacgttgtgaaagataatgaatcggtttgggctggtatcaattatagtgatagcgctaaaacttttgaaattaataacactaaagtcgaagttaaagccaaaggaatgtttattcttacaaagaaagatgataacacttatgaatgtagcttctataatcccgaatctacaaattccgtttcagatattgaatctaaaatttcaatgactggatactctattataaacaaaaatacgtcgacttctaatgaatccggcgtacgctttgaattaactaaataa

SEQ ID NO: 49 - protein, 412 aa, Staphylococcus aureus
IDSKNKPANSDIKFEVTQKSDAVKALKELPKSENVKNIYQDYAVTDVKTDKKGFTHYTLQPSVDGVHAPDKEVKVHADKSGKVVLINGDTDAKKVKPTNKVTLSKDDAADKAFKAVKIDKNKAKNLKDKVIKENKVEIDGDSNKYVYNVELITVTPEISHWKVKIDAQTGEILEKMNLVKEAAETGKGKGVLGDTKDININSIDGGFSLEDLTHQGKLSAFSFNDQTGQATLITNEDENFVKDEQRAGVDANYYAKQTYDYYKDTFGRESYDNQGSPIVSLTHVNNYGGQDNRNNAAWIGDKMIYGDGDGRTFTSLSGANDVVAHELTHGVTQETANLEYKDQSGALNESFSDVFGYFVDDEDFLMGEDVYTPGKEGDALRSMSNPEQFGQPAHMKDYVFTEKDNGGVHTNS

SEQ ID NO: 50 - DNA, 1239 bp, Staphylococcus aureus
  source 1..1239: mol_type = genomic DNA
attgattcaaaaaataaaccagctaattctgatattaaatttgaggtgactcaaaagagtgatgcggtcaaagcattaaaagaattgcctaaatccgaaaatgtaaaaaatatttatcaagattacgctgttactgatgtaaaaactgataaaaaaggatttacgcattatacattgcaaccgagtgttgatggtgttcatgcacctgacaaagaagtgaaagtacacgcagacaaatcaggaaaagtcgttttaatcaatggggatactgatgcgaagaaagtaaagccaacgaataaagtgacattaagtaaagatgacgcagccgacaaagcatttaaagcagttaagattgataagaataaagcgaaaaatcttaaagataaagtcattaaagaaaacaaagttgaaatcgatggtgacagtaataaatacgtttataatgttgagttaattacagtgacaccagaaatttcacattggaaagttaaaattgatgctcaaactggcgaaattttagaaaaaatgaacttagttaaagaagctgcagaaactggtaaaggaaaaggtgtacttggcgatacaaaagatatcaatatcaatagtattgacggtggatttagcctagaagatttaacgcatcaaggtaaattatcagcatttagctttaatgatcaaacaggtcaagcaacattgattactaatgaagatgaaaacttcgtaaaagatgagcaacgtgctggcgtagatgcaaattattacgctaaacaaacatatgattattacaaagacacatttggtcgtgaatcatatgacaaccaaggtagtccaattgtttcattaacgcatgttaataactacggtggtcaagataacagaaataatgccgcatggatcggtgacaaaatgatctatggtgatggtgatggtcgcacattcacaagtttatcgggtgcaaatgacgtagtagcacacgaattaacacacggtgtgacacaagagacagcgaacttagaatataaggaccagtcaggcgctctaaatgaaagcttttcagatgtttttggatactttgtagatgacgaggatttcttaatgggtgaagatgtctacacacctggaaaagagggagacgctttacgcagcatgtcaaacccagaacaatttggtcaaccagctcatatgaaagactatgtattcactgaaaaagataatggtggcgtacatacgaattcttaa

SEQ ID NO: 51 - RNA, 1239 nt, Staphylococcus aureus
  source 1..1239: mol_type = mRNA
attgattcaaaaaataaaccagctaattctgatattaaatttgaggtgactcaaaagagtgatgcggtcaaagcattaaaagaattgcctaaatccgaaaatgtaaaaaatatttatcaagattacgctgttactgatgtaaaaactgataaaaaaggatttacgcattatacattgcaaccgagtgttgatggtgttcatgcacctgacaaagaagtgaaagtacacgcagacaaatcaggaaaagtcgttttaatcaatggggatactgatgcgaagaaagtaaagccaacgaataaagtgacattaagtaaagatgacgcagccgacaaagcatttaaagcagttaagattgataagaataaagcgaaaaatcttaaagataaagtcattaaagaaaacaaagttgaaatcgatggtgacagtaataaatacgtttataatgttgagttaattacagtgacaccagaaatttcacattggaaagttaaaattgatgctcaaactggcgaaattttagaaaaaatgaacttagttaaagaagctgcagaaactggtaaaggaaaaggtgtacttggcgatacaaaagatatcaatatcaatagtattgacggtggatttagcctagaagatttaacgcatcaaggtaaattatcagcatttagctttaatgatcaaacaggtcaagcaacattgattactaatgaagatgaaaacttcgtaaaagatgagcaacgtgctggcgtagatgcaaattattacgctaaacaaacatatgattattacaaagacacatttggtcgtgaatcatatgacaaccaaggtagtccaattgtttcattaacgcatgttaataactacggtggtcaagataacagaaataatgccgcatggatcggtgacaaaatgatctatggtgatggtgatggtcgcacattcacaagtttatcgggtgcaaatgacgtagtagcacacgaattaacacacggtgtgacacaagagacagcgaacttagaatataaggaccagtcaggcgctctaaatgaaagcttttcagatgtttttggatactttgtagatgacgaggatttcttaatgggtgaagatgtctacacacctggaaaagagggagacgctttacgcagcatgtcaaacccagaacaatttggtcaaccagctcatatgaaagactatgtattcactgaaaaagataatggtggcgtacatacgaattcttaa

SEQ ID NO: 52 - DNA, 10 bp, synthetic construct
  source 1..10: mol_type = other DNA
attcggaacc

SEQ ID NO: 53 - DNA, 10 bp, synthetic construct
  source 1..10: mol_type = other DNA
atacgggacc